European Patent Application EP 4 563 589 A1, published June 4, 2025. Title: Antibacterial Protein Having Lytic Activity to Streptococci. Applicant: iNtRON Biotechnology, Inc. The sequence listing filed with the application follows.

SEQUENCE LISTING (2 sequences)

SEQ ID NO: 1 - protein, 279 aa, Artificial Sequence
MATYQEYKSRSNGNAYDIDGSFGAQCWDGYADYSKYLGLPYANCTNTGYARDIWEQRHENGILNYFDEVEVMQAGDVAIFMVVDGVTPYSHVAIFDSDAGGGYGWFLGQNQGGANGAYNIVKIPYSATYPTAFRPKVFKNAVTVTGNIGLNKGDYFIDVSARKPSSKAYYLANDVQLVNDIYQIKCDYLSPVGFDWTENGIPVSLVNWVDENGNHVPDGEDKDFKAGMYFSFEVDEVHITDTGDGGYYGGYYYRSFEFGQFGTVWLSVWDKDDLVNYYN

SEQ ID NO: 2 - DNA, 4907 bp, Artificial Sequence
  source 1..4907: mol_type = other DNA
aagaaaccaattgtccatattgcatcagacattgccgtcactgcgtcttttactggctcttctcgctaaccaaaccggtaaccccgcttattaaaagcattctgtaacaaagcgggaccaaagccatgacaaaaacgcgtaacaaaagtgtctataatcacggcagaaaagtccacattgattatttgcacggcgtcacactttgctatgccatagcatttttatccataagattagcggatcctacctgacgctttttatcgcaactctctactgtttctccatacccgtttttttgggctagaaataattttgtttaactttaagaaggagatatacatccatggctacgtatcaggagtataaatcgcggagcaatggcaacgcctatgatattgacggttcttttggtgcacagtgttgggacgggtatgcagactactctaaatatttggggctgccttacgccaactgtacaaacaccggttacgcccgtgatatctgggaacagcgtcacgagaatggcatcctgaactattttgacgaggtagaagtgatgcaagctggggatgttgcaatctttatggtggtggacggggttacaccatattcacacgtcgctatcttcgatagtgacgcaggtggcggctacggttggtttttaggccagaatcaagggggtgccaatggcgcctacaacatcgtcaaaattccttatagtgcaacatatcctactgcattccgtccaaaggttttcaaaaacgctgtcaccgttacaggcaatattgggttgaacaagggggactacttcattgacgtctcagcccgcaaacctagcagtaaagcgtactaccttgcaaacgacgttcaattagtgaatgacatttaccagatcaagtgcgactatctgtctccggttgggttcgattggaccgagaatggtattccagtatccttagtaaattgggtcgatgaaaacggcaatcacgtacctgatggtgaggataaagattttaaggccgggatgtatttctctttcgaggtagatgaggtacacattacagatacgggtgatggcggctattatggcggctattactatcgtagcttcgaattcgggcagtttgggacagtgtggttaagcgtttgggacaaagatgatctcgtaaactactataattaagcggccgcaagggcgagcttgaaggtaagcctatccctaaccctctcctcggtctcgattctacgcgtaccggtcatcatcaccatcaccattgagtttaaacggtctccagcttggctgttttggcggatgagagaagattttcagcctgatacagattaaatcagaacgcagaagcggtctgataaaacagaatttgcctggcggcagtagcgcggtggtcccacctgaccccatgccgaactcagaagtgaaacgccgtagcgccgatggtagtgtggggtctccccatgcgagagtagggaactgccaggcatcaaataaaacgaaaggctcagtcgaaagactgggcctttcgttttatctgttgtttgtcggtgaacgctctcctgagtaggacaaatccgccgggagcggatttgaacgttgcgaagcaacggcccggagggtggcgggcaggacgcccgccataaactgccaggcatcaaattaagcagaaggccatcctgacggatggcctttttgcgtttctacaaactcttttgtttatttttctaaatacattcaaatatgtatccgctcatgagattatcaaaaaggatcttcacctagatccttttaaattaaaaatgaagttttaaatcaatctaaagtatatatgagtaaacttggtctgacagttaggcgtcgcttggtcggtcatttcgaaccccagagtcccgctcagaagaactcgtcaagaaggcgatagaaggcgatgcgctgcgaatcgggagcggcgataccgtaaagcacgaggaagcggtcagcccattcgccgccaagctcttcagcaatatcacgggtagccaacgctatgtcctgatagcggtccgccacacccagccggccacagtcgatgaatccagaaaagcggccattttccaccatgatattcggcaagcaggcatcgccatgtgtcacgacgagatcctcgccgtcgggcatgcgcgccttgagcctggcgaacagttcggctggcgcgagcccctgatgctcttcgtccagatcatcctgatcgacaagaccggcttccatccgagtacgtgctcgctcgatgcgatgtttcgcttggtggtcgaatgggcaggtagccggatcaagcgtatgcagccgccgcattgcatcagccatgatggatactttctcggcaggagcaaggtgagatgacaggagatcctgccccggcacttcgcccaatagcagccagtcccttcccgcttcagtgacaacgtcgagcacagctgcgcaaggaacgcccgtcgtggccagccacgatagccgcgctgcctcgtcctgcagttcattcagggcaccggacaggtcggtcttgacaaaaagaaccgggcgcccctgcgctgacagccggaacacggcggcatcagagcagccgattgtcagttgtgcccagtcatagccgaatagcctctccacccaagcggccggagaacctgcgtgcaatccatcttgttcaatcatactcttcctttttcaatattattgaagcatttatcagggttattgtctcatgaccaaaatcccttaacgtgagttttcgttccactgagcgtcagaccccgtagaaaagatcaaaggatcttcttgagatcctttttttctgcgcgtaatctgctgcttgcaaacaaaaaaaccaccgctaccagcggtggtttgtttgccggatcaagagctaccaactctttttccgaaggtaactggcttcagcagagcgcagataccaaatactgtccttctagtgtagccgtagttaggccaccacttcaagaactctgtagcaccgcctacatacctcgctctgctaatcctgttaccagtggctgctgccagtggcgataagtcgtgtcttaccgggttggactcaagacgatagttaccggataaggcgcagcggtcgggctgaacggggggttcgtgcacacagcccagcttggagcgaacgacctacaccgaactgagatacctacagcgtgagctatgagaaagcgccacgcttcccgaagggagaaaggcggacaggtatccggtaagcggcagggtcggaacaggagagcgcacgagggagcttccagggggaaacgcctggtatctttatagtcctgtcgggtttcgccacctctgacttgagcgtcgatttttgtgatgctcgtcaggggggcggagcctatggaaaaacgccagcaacgcggcctttttacggttcctggccttttgctggccttttgctcacatgttctttcctgcgttatcccctgattctgtggataaccgtattaccgcctttgagtgagctgataccgctcgccgcagccgaacgaccgagcgcagcgagtcagtgagcgaggaagcggaagagcgcctgatgcggtattttctccttacgcatctgtgcggtatttcacaccgcatatggtgcactctcagtacaatctgctctgatgccgcatagttaagccagtatacactccgctatcgctacgtgactgggtcatggctgcgccccgacacccgccaacacccgctgacgcgccctgacgggcttgtctgctcccggcatccgcttacagacaagctgtgaccgtctccgggagctgcatgtgtcagaggttttcaccgtcatcaccgaaacgcgcgaggcagcagatcaattcgcgcgcgaaggcgaagcggcatgcataatgtgcctgtcaaatggacgaagcagggattctgcaaaccctatgctactccgtcaagccgtcaattgtctgattcgttaccaattatgacaacttgacggctacatcattcactttttcttcacaaccggcacggaactcgctcgggctggccccggtgcattttttaaatacccgcgagaaatagagttgatcgtcaaaaccaacattgcgaccgacggtggcgataggcatccgggtggtgctcaaaagcagcttcgcctggctgatacgttggtcctcgcgccagcttaagacgctaatccctaactgctggcggaaaagatgtgacagacgcgacggcgacaagcaaacatgctgtgcgacgctggcgatatcaaaattgctgtctgccaggtgatcgctgatgtactgacaagcctcgcgtacccgattatccatcggtggatggagcgactcgttaatcgcttccatgcgccgcagtaacaattgctcaagcagatttatcgccagcagctccgaatagcgcccttccccttgcccggcgttaatgatttgcccaaacaggtcgctgaaatgcggctggtgcgcttcatccgggcgaaagaaccccgtattggcaaatattgacggccagttaagccattcatgccagtaggcgcgcggacgaaagtaaacccactggtgataccattcgcgagcctccggatgacgaccgtagtgatgaatctctcctggcgggaacagcaaaatatcacccggtcggcaaacaaattctcgtccctgatttttcaccaccccctgaccgcgaatggtgagattgagaatataacctttcattcccagcggtcggtcgataaaaaaatcgagataaccgttggcctcaatcggcgttaaacccgccaccagatgggcattaaacgagtatcccggcagcaggggatcattttgcgcttcagccatacttttcatactcccgccattcagag